European Patent Specification EP 3 758 732 B1, published July 24, 2024. Title: PD-1 PEPTIDE INHIBITORS. Applicant: Leidos, Inc. The sequence listing filed with the application follows.

SEQUENCE LISTING (5 sequences)

SEQ ID NO: 1 - protein, 20 aa, Artificial Sequence
  artificial peptide
QTRTVPMPKIHHPPWQNVVP

SEQ ID NO: 2 - protein, 20 aa, Artificial Sequence
  artificial peptide
HHHQVYQVRSHWTGMHSGHD

SEQ ID NO: 3 - protein, 21 aa, Artificial Sequence
  artificial peptide
WNLPASFHNHHIRPHEHEWIQ

SEQ ID NO: 4 - protein, 20 aa, Artificial Sequence
  artificial peptide
SSYHHFKMPELHFGKNTFHQ

SEQ ID NO: 5 - protein, 9 aa, Plasmodium yoelii
SYVPSAEQI